European Patent Application EP 4 317 189 A1, published February 7, 2024. Title: MONOCLONAL ANTIBODY. Applicant: NATIONAL UNIVERSITY CORPORATION TOKAI NATIONAL HIGHER EDUCATION AND RESEARCH SYSTEM. The sequence listing filed with the application follows.

SEQUENCE LISTING (3 sequences)

SEQ ID NO: 1 - protein, 184 aa, Artificial Sequence
  VL OF CLONE 12G5A
MGHLKGRWSKMESQTQVLMSLLFWVSGTCGDIVMTQSPSSLTVTAGEKVTMSCKSSQSLLNSGNQKNYLTWYQQKPGQPPKLLIYWASTRESGVPDRFTGSGSGTDFTLTISSVQAEDLAVYYCQNDYSYPFTFGSGTKLEIKRADAAPTVSIFPPSSEQLTSGGASVVCFLNNFYPKDINVIF

SEQ ID NO: 2 - protein, 249 aa, Artificial Sequence
  VH OF CLONE 12G5A
MGWIWIFLFLLSGTAGVHSEVQLQQSGPELVKTGASVKISCKASGYSFTGYYMHWVKQSHGKSLEWIGYISCYNGATSYNQKFKGKATFTVDTSSSTAYMQFNSLTSEDSAVYYCARHYGNRYYAMDYWGQGTSVTVSSESQSFPNVFPLVSCESPLSDKNLVAMGCLARDFLPSTISFTWNYQNNTEVIQGIRTFPTLRTGGKYLATSQVLLSPKSILEGSDEYLVCKIHYGGKNRDLHVPIITRLEA

SEQ ID NO: 3 - protein, 339 aa, Homo sapiens
MSTVHEILCKLSLEGDHSTPPSAYGSVKAYTNFDAERDALNIETAIKTKGVDEVTIVNILTNRSNAQRQDIAFAYQRRTKKELASALKSALSGHLETVILGLLKTPAQYDASELKASMKGLGTDEDSLIEIICSRTNQELQEINRVYKEMYKTDLEKDIISDTSGDFRKLMVALAKGRRAEDGSVIDYELIDQDARDLYDAGVKRKGTDVPKWISIMTERSVPHLQKVFDRYKSYSPYDMLESIRKEVKGDLENAFLNLVQCIQNKPLYFADRLYDSMKGKGTRDKVLIRIMVSRSEVDMLKIRSEFKRKYGKSLYYYIQQDTKGDYQKALLYLCGGDD